European Patent Specification EP 3 704 221 B1, published April 10, 2024. Title: CLEANING COMPOSITIONS CONTAINING DISPERSINS II. Applicant: Henkel AG & Co. KGaA. The sequence listing filed with the application follows.

SEQUENCE LISTING (46 sequences)

SEQ ID NO: 1 - protein, 351 aa, GH20 catalytic domain from Actinobacillus pleuropneumoniae
MDLPKKESGLTLDIARRFYTVDTIKQFIDTIHQAGGTFLHLHFSDHENYALESSYLEQREENATEKNGTYFNPKTNKPFLTYKQLNEIIYYAKERNIEIVPEVDSPNHMTAIFDLLTLKHGKEYVKGLKSPYIAEEIDINNPEAVEVIKTLIGEVIYIFGHSSRHFHIGGDEFSYAVENNHEFIRYVNTLNDFINSKGLITRVWNDGLIKNNLSELNKNIEITYWSYDGDAQAKEDIQYRREIRADLPELLANGFKVLNYNSYYLYFVPKSGSNIHNDGKYAAEDVLNNWTLGKWDGKNSSNHVQNTQNIIGSSLSIWGERSSALNEQTIQQASKNLLKAVIQKTNDPKSH

SEQ ID NO: 2 - protein, 359 aa, GH20 catalytic domain from Aggregatibacter actinomycetemcomitans
CVKGNSIYPQKTSTKQTGLMLDIARHFYSPEVIKSFIDTISLSGGNFLHLHFSDHENYAIESHLLNQRAENAVQGKDGIYINPYTGKPFLSYRQLDDIKAYAKAKGIELIPELDSPNHMTAIFKLVQKDRGVKYLQGLKSRQVDDEIDITNADSITFMQSLMSEVIDIFGDTSQHFHIGGDEFGYSVESNHEFITYANKLSYFLEKKGLKTRMWNDGLIKNTFEQINPNIEITYWSYDGDTQDKNEAAERRDMRVSLPELLAKGFTVLNYNSYYLYIVPKASPTFSQDAAFAAKDVIKNWDLGVWDGRNTKNRVQNTHEIAGAALSIWGEDAKALKDETIQKNTKSLLEAVIHKTNGDE

SEQ ID NO: 3 - protein, 367 aa, GH20 catalytic domain from Actinobacillus succinogenes
DENDTAILQLQQTFRSAELSQNKETGLALDIARHFYPVEVIKAFIDTIHNAGGTFLHLHFSDHENYALESTVLNQRAENATRDKYGVYINPKTHKPFLSYAQLKDITDYAKNKNVELVPELDSPNHMTAIFDLLEKERGKPYTQQLRSKWTDEEIDITNPDSIAFIKSLIAEVIEIFGDSSRHFHIGGDEFGYGTDNNHEFITYVNTLAEFLQQKGLKTRIWNDGLIKATIHQLNPDIQITYWSYDGNPQDEQEERRRREIRMSMPELIAQGFAVLNYNAYYLYFTPQEDATTSHDSNFATRDVLKNWDLTIWDGQNSQNKIRDRHKIMGSALSIWGEKAGSLRSDSIQKYTAPLLTAIIYKSKITG

SEQ ID NO: 4 - protein, 349 aa, GH20 catalytic domain from Neisseria wadsworthii
QSVAPKQGGLMLDTARHFYPTNVIKDFIDTIAKSGGNFLHLHFSDHENYALESHILNQRAADATRNADGVYINPVTGKPFLSFEQLEEIKAYAKSKNIELIPEVDSPNHMTTIFTLLEAHRGKDFVNKIKSKYSDEEINITNPESIAFMKSLIGEVADAFGDSSRHFHIGGDEFGYSVDSNHEFIAYANDLSAFLKQKGLTTRIWNDGIIKATVDKLNPEIQVTYWSYDGDVQNKQASQERRRIRTSMPDLIEKGFSVLNYNSYYLYVNPKQEWGTSYNSDFATRDIINRWNLGVWDGENQQNAVKNTDKIMGAALAIWGENAGSMSSKTIQKYTAGLLESIIRKTHAE

SEQ ID NO: 5 - protein, 352 aa, GH20 catalytic domain from Actinobacillus capsulatus
MNHSQIKEAGLTLDIARRFYPVETIKQFIDTIHHAGGTFLHLHFSDHENYALESTYLDQLEANAIVKDGTYYNPTTNKPFLTYKQINDIIYYAKSKNIELVPEVDTPNHMTAIFRLLEAKHSKDYVKRLKSKMNDEEIDITNLESIEVIKTLIAEVIYIFGHASEHFHIGGDEFGYSVETNHEFITYVNTLNQFINNKGKITRIWNDGLIKNNLNQLNKNVEITYWSYDGDAQESQDIAERRKIRVNLPELLENGFKVLNYNSYYLYFVPKGNANITHDSKHATEDVLKNWKLGLWDGQNKENIVENTKNIIGSSLSIWGEHSGSLSSAVIEESTQELLKAVIQKTNDPKSH

SEQ ID NO: 6 - protein, 324 aa, GH20 catalytic domain from Terribacillus goriensis
QDQEKGITIDISRKYYSIETLKSIIDEISANGGDYLQLHFSDNERYAIASEFLGQNGENPNSTYLTKKELLSLIAYSNDRDIMVIPDIDLPAHSRGWLNIMKEKDSGLYTDIVTDYSEDTLDYHNNAVALYTANQLLDEVLDLFYQPKFAGKQRIVLGGDEVPGSGVHQTDFIRFMNQIAETAKASNYKPQMWNDSITPEGIQNLDRSFSILYWKQSTLSNGAQGLDVQDFEENGLSVYNYNAYSLYFLPATRFTQEDITEQIDYMKWAYAYNKFFYISDYYKQVDTSNVKGSSLVFWGEHANDLSQEGLLKQEKPLIQNFLGL

SEQ ID NO: 7 - protein, 324 aa, GH20 catalytic domain from Terribacillus saccharophilus
QDQEKGITIDISRKYYSIKTLKAIVDEISANGGDYLQLHFSDNESYAIASEFLGQNSENPNSAYLTKKELLSLIAYSNDRNIMVIPDIDLPAHSKGWLNIMKEKDSGLYTDIVTDYSEDTLDYHNNAVALYTANQLLDEVLDLFYQPKFAGKQRIVLGGDEVPGSGAHQTDFIRFMNQIAKTAKASNYEPQMWNDSITPEGIQNLDRSFSILYWKQSTLSNGAQSLDVQDFEENGLSVYNYNAYSLYFLPSTRFTQEDITEQIDYMKWAYAYNKFFYISDYYKQVDTPNVKGSSLVFWGEHANDLSQEGLLKQEKPLIQNFLGL

SEQ ID NO: 8 - protein, 325 aa, GH20 catalytic domain from Curtobacterium oceanosedimentum
ETGVMLDVARAYYPVSLIEQYVDLLAEHGGGFLHLHLTDDQNVGIESAVLGQTPANAVLRNGVYTSRVTGRPFLSAAQARAISAYAAKRGIAIVPEVDSPGHMAAAFALLEARHGATWVDRIRSGESELDTSVPESATLAAELLREVTQTFPSSRTVHIGGDEWGADVSADERVGWMNAMAAAIGDREVWAWNDGIDRASVGRLDPRIHVTYWSFDGDTEDAAERRERRARRASATDLQRAGIDLLNYNSYYLYEVPTDLDPADSEYTVADLREHWSLRAWDGDSGARLAAPMSGAAVAIWGEDLDGAPSEALLRWSAPHVTAMI

SEQ ID NO: 9 - protein, 378 aa, full length polypeptide from Actinobacillus capsulatus
MKKIISLLTLIFIGLLSSCSSSTVNAMNHSQIKEAGLTLDIARRFYPVETIKQFIDTIHHAGGTFLHLHFSDHENYALESTYLDQLEANAIVKDGTYYNPTTNKPFLTYKQINDIIYYAKSKNIELVPEVDTPNHMTAIFRLLEAKHSKDYVKRLKSKMNDEEIDITNLESIEVIKTLIAEVIYIFGHASEHFHIGGDEFGYSVETNHEFITYVNTLNQFINNKGKITRIWNDGLIKNNLNQLNKNVEITYWSYDGDAQESQDIAERRKIRVNLPELLENGFKVLNYNSYYLYFVPKGNANITHDSKHATEDVLKNWKLGLWDGQNKENIVENTKNIIGSSLSIWGEHSGSLSSAVIEESTQELLKAVIQKTNDPKSH

SEQ ID NO: 10 - protein, 349 aa, full length polypeptide from Terribacillus goriensis
MLIKFLSITTVSILLFLTMSNTAQAQDQEKGITIDISRKYYSIETLKSIIDEISANGGDYLQLHFSDNERYAIASEFLGQNGENPNSTYLTKKELLSLIAYSNDRDIMVIPDIDLPAHSRGWLNIMKEKDSGLYTDIVTDYSEDTLDYHNNAVALYTANQLLDEVLDLFYQPKFAGKQRIVLGGDEVPGSGVHQTDFIRFMNQIAETAKASNYKPQMWNDSITPEGIQNLDRSFSILYWKQSTLSNGAQGLDVQDFEENGLSVYNYNAYSLYFLPATRFTQEDITEQIDYMKWAYAYNKFFYISDYYKQVDTSNVKGSSLVFWGEHANDLSQEGLLKQEKPLIQNFLGL

SEQ ID NO: 11 - protein, 365 aa, full length polypeptide from Terribacillus saccharophilus
MVSRTMLFIKREKGKTVLIKFLSITTVSILLFLTMANTAQAQDQEKGITIDISRKYYSIKTLKAIVDEISANGGDYLQLHFSDNESYAIASEFLGQNSENPNSAYLTKKELLSLIAYSNDRNIMVIPDIDLPAHSKGWLNIMKEKDSGLYTDIVTDYSEDTLDYHNNAVALYTANQLLDEVLDLFYQPKFAGKQRIVLGGDEVPGSGAHQTDFIRFMNQIAKTAKASNYEPQMWNDSITPEGIQNLDRSFSILYWKQSTLSNGAQSLDVQDFEENGLSVYNYNAYSLYFLPSTRFTQEDITEQIDYMKWAYAYNKFFYISDYYKQVDTPNVKGSSLVFWGEHANDLSQEGLLKQEKPLIQNFLGL

SEQ ID NO: 12 - protein, 485 aa, full length polypeptide from Curtobacterium oceanosedimentum
MIAGAVVVVTAAAVLVGVGAVAGPADRNTSAAEAAVTSIAPRATITGVAAISAATSSRTTVRTTLTLENRSGERESAADAWLYLAGGGARYALGHAPVRALAAGARATVRTTLRVPSRAPAGKYAVLACAGPYSKQACRTSGTTVTVGTAARARPETGVMLDVARAYYPVSLIEQYVDLLAEHGGGFLHLHLTDDQNVGIESAVLGQTPANAVLRNGVYTSRVTGRPFLSAAQARAISAYAAKRGIAIVPEVDSPGHMAAAFALLEARHGATWVDRIRSGESELDTSVPESATLAAELLREVTQTFPSSRTVHIGGDEWGADVSADERVGWMNAMAAAIGDREVWAWNDGIDRASVGRLDPRIHVTYWSFDGDTEDAAERRERRARRASATDLQRAGIDLLNYNSYYLYEVPTDLDPADSEYTVADLREHWSLRAWDGDSGARLAAPMSGAAVAIWGEDLDGAPSEALLRWSAPHVTAMIETAAS

SEQ ID NO: 13 - DNA, 1134 bp, codon optimized gene from Actinobacillus capsulatus
atgaagaagatcatctctcttcttacgcttatcttcatcggccttctttcttcttgctcatcatctacagtaaacgcgatgaaccactctcaaatcaaggaagctggccttactttagacattgctcgtcgcttctacccagttgagacaatcaagcaattcatcgacactatccaccatgctggtggcacattccttcaccttcacttctcagaccacgagaactacgcgcttgagtctacgtaccttgaccaacttgaggcgaacgcgatcgttaaggacggcacatactacaacccaacgacaaacaagcctttccttacttacaagcaaatcaacgacatcatctactacgcgaagtctaagaacatcgagcttgtacctgaggtagacacaccgaaccacatgacagcgatcttccgccttcttgaggcgaagcacagcaaggactacgtaaagcgccttaagtcaaagatgaacgacgaggagatcgacatcactaaccttgagtctatcgaggttatcaagactcttatcgctgaggttatctacatcttcggccacgcgagcgagcacttccacattggtggcgacgagttcggctactcagttgagacgaaccacgagttcatcacttacgttaacacgcttaaccagttcatcaacaacaagggcaagatcacgcgcatctggaacgacggccttatcaagaacaaccttaaccaacttaacaagaacgttgagatcacgtactggtcttacgacggcgacgcgcaagagtcacaagacatcgcggaacgtcgcaagatccgcgtaaaccttcctgagcttcttgagaacggcttcaaggttcttaactacaactcttactacctttacttcgtacctaagggcaacgcgaacatcacgcacgactctaagcacgcgactgaggacgttcttaagaactggaagcttggcctttgggacggccaaaacaaggagaacatcgttgagaacacgaagaacatcatcggctcatctctttctatctggggtgagcactctggctcactttcatctgcggttatcgaggagtctacgcaagagcttcttaaggcggttatccaaaagacaaacgacccaaagtctcac

SEQ ID NO: 14 - DNA, 1047 bp, codon optimized gene from Terribacillus goriensis
atgcttatcaagttcctttctatcacgacagtttcaatccttcttttccttacgatgtctaacactgcgcaagcgcaagaccaagagaagggcatcacaatcgacatctctcgcaagtactactctatcgagacacttaagtctatcatcgacgagatctcagcgaatggtggcgactaccttcaacttcatttctctgacaacgagcgctacgcgatcgcgtcagagttccttggccaaaacggcgagaacccaaactctacttaccttacaaagaaggagcttctttctcttatcgcgtactctaacgaccgcgacatcatggtaatcccagacatcgaccttccagcgcattctcgtggctggcttaacatcatgaaggagaaggactcaggcctttacactgacatcgtaacggactactctgaggacacacttgactaccataacaacgctgtagcgctttacacagcaaaccaacttcttgacgaggtacttgaccttttctaccaaccgaagtttgctggcaagcagcgcatcgtacttggtggcgacgaggttcctggctctggcgtacaccagactgacttcatccgcttcatgaaccaaatcgcggagactgcgaaggcttctaactacaagccacaaatgtggaacgactctatcacacctgagggcatccaaaaccttgaccgctcattctctatcctttactggaagcaatctacacttagcaatggtgcgcaaggccttgacgtacaagacttcgaggagaacggccttagcgtttacaactacaatgcgtactcactttacttccttcctgcgacacgcttcactcaagaggacatcactgagcaaatcgactacatgaagtgggcgtatgcgtacaacaagttcttctacatctctgactactacaagcaagtagacacaagcaacgttaagggctcttctcttgtattctggggtgagcatgcgaacgaccttagccaagagggccttcttaagcaagagaagccacttatccaaaacttccttggcctt

SEQ ID NO: 15 - DNA, 1095 bp, codon optimized gene from Terribacillus saccharophilus
atggtatctcgcacgatgcttttcatcaagcgcgagaagggcaagacggttcttatcaagttcctttctatcacgacagtatctatccttcttttccttacgatggcgaacactgcgcaagcgcaagaccaagagaagggcatcacaatcgacatctctcgcaagtactacagcatcaagacgcttaaggcgatcgttgacgagatctcagcgaatggtggcgactaccttcaacttcacttctctgacaacgagagctacgcgatcgcgtctgagttccttggccaaaactctgagaacccaaactctgcgtaccttacaaagaaggagcttctttcacttatcgcgtactctaacgaccgcaacatcatggttatcccggacatcgaccttcctgcgcactcaaagggctggcttaacatcatgaaggagaaggactctggcctttacacagacatcgtaactgactactcagaagacactcttgactaccacaacaacgcggttgcgctttacacggcgaaccaacttcttgacgaggttcttgaccttttctaccaacctaagtttgctggcaagcaacgcatcgttcttggtggcgacgaggttcctggctctggtgcgcaccaaactgacttcatccgcttcatgaaccagatcgcgaagacagcgaaggcgtctaactacgagccacaaatgtggaacgacagcatcactcctgagggcatccaaaaccttgaccgctctttctctatcctttactggaagcaatcaacgctttcaaatggtgcgcaatctcttgacgtacaagacttcgaggagaacggcctttcagtttacaactacaacgcttacagcctttacttccttcctagcactcgcttcacgcaagaggacatcacggagcaaatcgactacatgaagtgggcgtatgcgtacaacaagttcttctacatctctgactactacaagcaagtagacacaccaaacgtaaagggctcatctcttgtattctggggtgagcacgcgaacgacctttctcaagagggccttcttaagcaagagaagccacttatccaaaacttccttggcctt

SEQ ID NO: 16 - DNA, 1455 bp, codon optimized gene from Curtobacterium oceanosedimentum
atgatcgctggtgcggtagttgtagttacagcggctgctgttcttgttggcgttggtgctgttgctggccctgcagaccgcaatacttctgctgcggaagctgcggtaacgtcaatcgctccgcgtgcaactattacaggagttgcagcaatctctgctgctactagctcacgtacaacagttcgcactactttaacattagaaaaccgttctggtgagcgtgaatctgcagctgatgcttggctttatcttgcaggaggcggagctcgttatgctcttggtcatgctcctgttcgcgcacttgcagctggagctcgtgctacagttcgcacaacacttcgcgttccatcacgtgcgcctgctggcaaatacgctgttcttgcttgtgccggaccatactctaaacaagcatgtcgcactagcggtactactgttacagttggcactgcggctcgtgctcgccctgagacgggagttatgttagatgttgctcgtgcgtattacccggttagccttatcgaacagtacgttgatttgcttgcagaacatggtggtggctttttgcatttacatcttactgacgaccaaaatgttggtattgaatctgcggtacttggccaaacacctgctaacgctgtacttcgtaatggcgtatacacttctcgtgttactggtcgtcctttcttatctgctgcgcaagctcgtgctattagcgcttatgctgctaaacgtggtattgcgatcgttcctgaggttgattctccaggacacatggctgcagcttttgcacttttagaggcacgccatggtgctacatgggttgatcgtatccgttctggtgagtcagaattagacacttctgttccggaatcagctacgttagcggcagaattgcttcgtgaagtaactcagactttcccaagctctcgtactgttcacattggtggtgacgaatggggagcagacgtttctgctgacgagcgcgttggttggatgaacgctatggctgctgctatcggtgaccgtgaagtttgggcatggaacgacggcatcgatcgcgctagcgtaggtcgtttagatccacgtattcatgtaacttattggtcattcgacggtgacactgaagatgcagcggaacgtcgtgagcgtcgcgcacgccgtgcatctgccacagatcttcaacgtgctggaattgaccttcttaactacaacagctattacttatacgaagtacctactgacttagaccctgcggattctgagtatacagttgcagatcttcgtgaacactggagccttcgtgcatgggacggagactctggagctcgcttagcagctcctatgagcggtgctgcagttgcgatctggggtgaggaccttgatggcgctccatctgaagcattgttgcgttggtcagcaccacacgttactgcaatgatcgagactgctgcatca

SEQ ID NO: 17 - protein, 352 aa, mature polypeptide from Actinobacillus capsulatus; identical to SEQ ID NO: 5

SEQ ID NO: 18 - protein, 324 aa, mature polypeptide from Terribacillus goriensis; identical to SEQ ID NO: 6

SEQ ID NO: 19 - protein, 324 aa, mature polypeptide from Terribacillus saccharophilus; identical to SEQ ID NO: 7

SEQ ID NO: 20 - protein, 461 aa, mature polypeptide sequence from Curtobacterium oceanosedimentum
ADRNTSAAEAAVTSIAPRATITGVAAISAATSSRTTVRTTLTLENRSGERESAADAWLYLAGGGARYALGHAPVRALAAGARATVRTTLRVPSRAPAGKYAVLACAGPYSKQACRTSGTTVTVGTAARARPETGVMLDVARAYYPVSLIEQYVDLLAEHGGGFLHLHLTDDQNVGIESAVLGQTPANAVLRNGVYTSRVTGRPFLSAAQARAISAYAAKRGIAIVPEVDSPGHMAAAFALLEARHGATWVDRIRSGESELDTSVPESATLAAELLREVTQTFPSSRTVHIGGDEWGADVSADERVGWMNAMAAAIGDREVWAWNDGIDRASVGRLDPRIHVTYWSFDGDTEDAAERRERRARRASATDLQRAGIDLLNYNSYYLYEVPTDLDPADSEYTVADLREHWSLRAWDGDSGARLAAPMSGAAVAIWGEDLDGAPSEALLRWSAPHVTAMIETAAS

SEQ ID NO: 21 - protein, 9 aa, Artificial
  conserved motif I
  misc_feature (1)..(1): Xaa = I (Ile) or V (Val)
  misc_feature (3)..(3): Xaa = E (Glu) or D (Asp)
  misc_feature (4)..(4): Xaa = L (Leu) or V (Val) or I (Ile)
  misc_feature (6)..(6): Xaa can be any naturally occurring amino acid
  misc_feature (8)..(8): Xaa = A (Ala) or N (Asn)
XPXXDXPXH

SEQ ID NO: 22 - protein, 8 aa, Artificial
  conserved motif II
  MISC_FEATURE (4)..(4): Xaa = A(Ala) or S (Ser)
  MISC_FEATURE (6)..(6): Xaa = S (Ser) or Y (Tyr)
NYNXYXLY

SEQ ID NO: 23 - protein, 27 aa, Artificial
  Bacillus clausii secretion signal
MKKPLGKIVASTALLISVAFSSSIASA

SEQ ID NO: 24 - protein, 8 aa, Artificial
  His-Tag
HHHHHHPR

SEQ ID NO: 25 - protein, 486 aa, Full length polypeptide from Curtobacterium flaccumfaciens
MVRQQGNVGPGSSARRTLAVGLAIALSAAALVGIRATAGSADTAVSAVTVTKVTASTTGTVVRTTLKVENTAPVRKPASSVWLYLSAGTEKYTLGRVAVKALAAGSSTSVTAVRGTPSRAAAGKYSVLACAGAYSAKQCRTSTATVTTKPTKRARPETGVMLDVARAYYPVALIKRYIDLLADDGGRFLHLHLTDDQNVGIESTVLGQTPANADLDHGVYTSRVTHRPFLSAAQARTISAYGAERGVAIVPEIDTPGHMAAAFALLEAQHGTKWVDRIRSGENELDTSAPESLALAKKLYAEVQRTFPSSRTVHIGGDEWGDDVTAAQRVTWMNAMAAALDDREVWAWNDGIDRVAVGRLDPRIHVTYWSFDGDTEDAAERRERRARRASAVDLQQAGIDQLNYNSYYLYEVPTDLDPADSDYTVADLRENWSLRAWDGDSGSLLAAPMSGAAVAIWGEDLEDPPSDALLRWSAPHVTAMIETAAS

SEQ ID NO: 26 - protein, 486 aa, full length polypeptide from Curtobacterium luteum
MVRQQGNVGPGSSARRTLAVGLAIALSAAALVGIRATAGSADTAVSAVTVTKVTASTTGTAVRTTLKVENTAPVRKPASSVWLYLSAGTEKYTLGRVAVKALSAGSSTSVTAVRGTPSRAAAGKYWVLACAGAYSAKQCRTSTATVTTKPTKRARPETGVMLDVARAYYPVALIKRYIDLLADDGGRFLHLHLTDDQNVGIESTVLGQTPANADLDHGVYTSRVTHRPFLSAAQARTISEYGAERGVTIVPEIDTPGHMAAAFALLEAQHGTKWVDRIRSGENELDTSAPESLVLAKKLYAEVQRTFPSSRTVHIGGDEWGDDVTAAHRVAWMNEMAATLGNREVWAWNDGIDRVAVGRLDPRIHVTYWSFDGDTEDAAERRERRARRASAVDLQQAGIDQLNYNSYYLYEVPTDLDPADSDYTVADLRENWSLRAWDGDSGSLLAAPMSGAAVAIWGEDLEDPPSDALLRWSAPHVTAMIETAAS

SEQ ID NO: 27 - protein, 481 aa, Full length polypeptide from Curtobacterium oceanosedimentum
MKRSIAVGLVIAMSAAVVIGADAIGGSAGTADASGAPRLVVTKVTASSTTTSTRTTVRTTLTVKNTSVARKPAADAWLSLTAGSKRYTLGHVSVQSLAAGASATIHATHTAPPRAPAGKYAVLACTGAFSLSKCGTSATTVTTARATRARPDTGVMLDVARAYYPVALIEQYIALLADHGGRFLHLHLTDDQNVGIESEVLGQTLANADLRDGVYTSRITGRPFLSAAQAREISRYAAQRGIAIIPEIDTPGHMAAAFALLEAGHGKQWVDRIRSGESELDTSAPGSSALAARLLQEVTRTFPSSRTVHIGGDEWGDDVTADERVQWLNTMAAAVGNRAVWAWNDGIDRAAIGRLDPRIHVTYWSFDGDTEDATERRERRERRAGANDLYAAGIDLLNYNSYYLYEVPTDLDAADSEYTVADLRENWSLRTWDGDSGARLAGPTSGAAVAIWGEDLEAPPSDALLRWSAPHVLAMIETAGS

SEQ ID NO: 28 - protein, 475 aa, Full length polypeptide from Curtobacterium Leaf154
MVAAGLAIAVSAAALIGIDVIAGSAAGSTTSTVTVTQVTATTTASSTGTAVRTTLKIKNTAAVRKPASSAWLYLSAGTKKYTLGRVAVKALAAGSSTSVTAVRGTPSRATAGEYSVLACAGAYSAKQCRTSTATVTTKPTKRARPETGVMLDVARAYYPVALIKRYIDLLADDGGRFLHLHLTDDQNVGIESTVLGQTLANADLDEGVYTSRVTRRPFLSAAQARTISDYAARRGVAIVPEIDTPGHMTAAFDLLEAQHGTKWVDRIRSGENELDTSTPGSLALAKKLYAEVQRTFPASRTVHIGGDEWGDDVSAAERVAWMNAMAAALGNREVWAWNDGIDRVAVGRLDPRIHVTYWSFDGDTEDAAERRERRARRASAVDLQQAGIDMLNYNSYYLYEVPTDLDPADSEYTVADLRENWSLRTWDGDSGSLLAAPMSGAAVAIWGEDLEDPPSDALLRWSAPHVTAMIETAAS

SEQ ID NO: 29 - DNA, 1461 bp, Curtobacterium flaccumfaciens
gtggtgcgtcagcaggggaacgtgggtcccggatcgtctgccagacgcacgcttgcggtcggtctggcgatcgccctgtcggccgcagctctggtcggcatccgtgcaacggcaggatcagcggacaccgcagtctcggcggtgacggtcacgaaggtcaccgcgtccaccaccggcaccgttgtgcgcaccaccctgaaggtcgagaacaccgccccggtgcggaagccggcctcctccgtgtggctgtacctgtccgccggcaccgagaagtacacgctcggccgggtcgcggtgaaggcactcgccgctggttcgagcacctcggtcaccgcagtccgcgggacaccttcccgtgccgcagccggcaagtactcggtcctcgcctgcgccggtgcgtactccgcgaagcagtgccgcacgtcgacggcgaccgtcaccaccaagcccacgaagcgcgcgcgtccggagacgggcgtgatgctcgacgtcgctcgcgcctactaccccgtggcgttgatcaagcggtacatcgacctcctcgccgacgacggcgggcgcttcctgcacctgcacctcaccgatgaccagaacgtcgggatcgagagcacggtcctcggccagacccccgcgaacgcggatctcgaccacggcgtctacaccagccgcgtgacccatcgtccgttcctgagcgccgcgcaggcacgcacgatctccgcgtacggggccgagcgaggcgtcgcgatcgtgccggagatcgacacccccggacacatggccgccgcgttcgccctgctcgaggcgcagcacggcacgaagtgggtcgaccgcatccgttcgggcgagaacgagctcgacacgtcggcgcccgagagtctcgccctggcgaagaagctgtacgcagaggtgcagcggaccttcccctccagccgaaccgtgcacatcggcggtgatgaatggggcgacgacgtcaccgccgcccaacgcgtcacctggatgaacgcgatggcggccgcgctcgacgaccgcgaggtgtgggcctggaacgacgggatcgatcgggtcgcggtcgggcgactcgatccgcgcatccacgtcacgtactggagcttcgacggcgacaccgaggacgcagcagaacggcgcgaacgccgagcgcggcgggcgagtgcggtcgacctgcagcaggccgggatcgaccagctcaactacaactcgtactacctctacgaggtgccgaccgacctcgacccggccgacagcgattacacggtcgccgatctccgcgagaactggtcgctccgggcgtgggacggcgactccggttcgcttctcgcggctccgatgtcgggcgccgccgtcgcgatctggggtgaggacctcgaagacccgccatccgacgcgctcctgcggtggagcgcaccgcacgtgacggcgatgatcgagaccgcagcctcctga

SEQ ID NO: 30 - DNA, 1461 bp, Curtobacterium luteum
gtggtgcgtcagcaggggaacgtgggtcccggatcgtctgccagacgcacgcttgcggtcggtctggcgatcgccctgtcggccgcagctctggtcggcatccgtgcaacggcaggatcagcggacaccgcagtctcggcggtgacggtcacgaaggtcaccgcgtccaccaccggcaccgctgtgcgcacaaccctgaaggtcgagaacaccgccccggtgcggaagccggcctcctccgtgtggctgtacctgtccgccggcaccgagaagtacacgctcggccgggtcgcggtgaaggcgctgtcggctggttcgagcacctcggtcaccgcagtccgcgggacaccttcccgtgccgcagccggcaagtactgggtcctcgcctgcgccggtgcgtactccgcgaagcagtgccgcacgtcgacggcgaccgtcaccaccaagcccacgaagcgcgcgcgtccggagacgggcgtgatgctcgacgtcgctcgcgcctactaccccgtggcgttgatcaagcggtacatcgacctcctcgccgacgacggcgggcgcttcctgcacctgcacctcaccgatgaccagaacgtcgggatcgagagcacggtcctcggccagactcccgcgaacgcggatctcgaccacggcgtctacaccagccgcgtgacccatcgcccgttcctgagtgccgcgcaggcacgcacgatctccgagtacggggcggagcgaggcgtcacgatcgtgccggagatcgacactcccggacacatggccgccgcgttcgccctgctcgaggcgcagcacggcacgaagtgggtcgaccgcatccgttcgggcgagaacgagctcgacacgtcggcgcccgagagtctcgtgctggcgaagaagctgtacgcagaggtgcagcggaccttcccttccagccgaaccgtgcacatcggcggcgacgaatggggcgacgacgtcaccgccgcacatcgcgtcgcctggatgaacgagatggcggccacgctcggcaaccgcgaggtctgggcctggaacgacgggatcgatcgggttgcggtcgggcgactcgatccgcgcatccacgtcacgtactggagcttcgacggcgacaccgaggacgcagcagaacggcgcgaacgccgagcgcggcgggcgagtgcggtcgacctgcagcaggccgggatcgaccagctcaactacaactcgtactacctctacgaggtgccgaccgacctcgacccggccgacagcgattacacggtcgccgatctccgcgagaactggtcgctccgggcgtgggacggcgactccggttcgcttctcgcggctccgatgtcgggcgccgccgtcgcgatctggggtgaggacctcgaagacccgccatccgacgcgctcctgcggtggagcgcaccgcacgtgacggcgatgatcgagaccgcagcctcctga

SEQ ID NO: 31 - DNA, 1446 bp, Curtobacterium oceanosedimentum
gtgaagcgcagcatcgccgtcggcctggtgatcgcgatgtcggcggcagtcgtgatcggagcggacgcgatcggcggatcggcgggcactgctgatgcgtccggagctccgcggctggtggtcaccaaggtcaccgcgagcagcaccaccacgtcgacacgcaccacggtgcgcacgacgctgacggtcaagaacacctcggtggcgcgcaagccggcggccgacgcatggctctccctgacggccgggagcaagcggtacaccctcggacacgtctcggtgcagtcactcgctgccggtgcgagcgcgacgatccacgcgacgcacaccgcgcctcctcgtgcgccggccgggaagtacgcggtcctcgcgtgcacgggagccttctccctgtcgaagtgcggcacctcggccacgaccgtcaccaccgcccgtgcgacccgggcacgtcccgacaccggcgtgatgctcgacgtggctcgtgcctactacccggtggcgctgatcgagcagtacatcgcgctcctcgctgatcacggtggtcgcttcctgcacctccacctcaccgacgaccagaacgtgggcatcgagagcgaggtcctcggccagaccctcgcgaacgccgatctccgggacggcgtctacacgagtcggatcaccggtcggccgttcctcagcgcggcgcaggcacgggagatctcccggtacgccgcgcaacgaggcatcgcgatcattcccgagatcgacacccccggtcacatggctgcggcgttcgctctcctcgaggccggacacggcaagcagtgggtggaccggatccgttcgggcgagagcgaactcgacacgtcggcgcccggcagctccgcgctggcggcacgactcctgcaggaggtcacgcggaccttcccgtcgagccgcaccgtccacatcggcggcgacgagtggggcgacgacgtcaccgccgacgaacgcgtccagtggttgaacacgatggcggccgccgtcggcaaccgtgcggtgtgggcgtggaacgacgggatcgaccgggctgcgatcgggcgactggatccgcgtatccacgtcacctactggagcttcgacggtgacaccgaggacgcgacggaacgccgcgagcgccgcgagcgacgggcgggtgcgaacgacctgtacgcggccgggatcgacctgctgaactacaactcgtactacctgtacgaggtgccgacggacctcgatgcggccgacagcgagtacaccgtcgccgatctccgcgagaactggtcgctccggacctgggacggggactcgggcgcacgtctggcgggtccgacgtcgggggcggccgtcgcgatctggggcgaggacctcgaagcgccaccgtccgacgcgctcctgcgctggagcgccccacacgtgctcgcgatgatcgagaccgccggctcgtag

SEQ ID NO: 32 - DNA, 1428 bp, Curtobacterium leaf154
atggtcgcagccggtctggcgatcgcggtgtctgcggcagccctgatcggcatcgatgtgatcgccgggtcagctgccgggtcgaccacctcgacggtgacggtcacccaggtcaccgcgacgaccaccgccagctccaccggcaccgccgttcgcaccaccctcaagatcaagaacactgccgccgtgcggaagccggcttcctccgcttggctgtacctgtccgccggcacgaagaagtacacactcggccgggtcgcggtgaaggcactcgccgctggttcgagcacgtccgtcaccgcagtccgcgggacgccctcccgtgccacggccggcgagtactcggtcctcgcctgcgccggtgcgtactcggcgaagcagtgccgcacgtcgaccgcgaccgtcaccaccaagccgacgaagcgcgcgcgtccggagacgggcgtgatgctcgacgtcgctcgcgcctactaccccgtggcgctgatcaagcggtacatcgacctgctcgccgacgacggtgggcgcttcctgcacctgcacctcaccgatgaccagaacgtcgggatcgagagcacggtgctcggccagaccctcgccaacgctgatctcgacgaaggcgtgtacacgagccgtgtgacccgtcgtccgttcctgagcgccgcgcaggcacgcaccatctccgactacgcagcgaggcggggtgtcgcgatcgtgcccgagatcgacactccgggccacatgactgcggcattcgacctgctcgaggcgcagcacggcacgaagtgggtcgaccgcatccgttcgggcgagaacgaactcgacacgtcgacgcccgggagcctcgcgctggcgaagaagctgtacgcagaggtgcagcggaccttccccgccagccgaaccgtgcacatcggcggtgatgagtggggcgacgacgtctcggccgccgaacgggtcgcgtggatgaacgcgatggcggccgctctcggcaaccgcgaggtctgggcctggaacgacgggatcgatcgggtcgcggtcgggcgactggacccgcgcatccacgtcacgtactggagcttcgacggcgacaccgaggacgcagccgagcggcgcgaacggcgagcgcgacgggcgagtgcggtcgacctgcagcaggccgggatcgacatgctcaactacaactcgtactacctgtacgaggtaccgaccgacctcgacccggccgacagcgagtacaccgtcgccgatctccgcgagaactggtcactccggacgtgggacggcgactccggttcgctgctcgcggctccgatgtcgggcgccgccgtcgcgatctggggtgaggacctcgaagacccgccatctgacgcgctcctgcggtggagcgcaccgcacgtgacggcgatgatcgagaccgcagcctcctga

SEQ ID NO: 33 - protein, 445 aa, mature polypeptide from Curtobacterium flaccumfaciens
DTAVSAVTVTKVTASTTGTVVRTTLKVENTAPVRKPASSVWLYLSAGTEKYTLGRVAVKALAAGSSTSVTAVRGTPSRAAAGKYSVLACAGAYSAKQCRTSTATVTTKPTKRARPETGVMLDVARAYYPVALIKRYIDLLADDGGRFLHLHLTDDQNVGIESTVLGQTPANADLDHGVYTSRVTHRPFLSAAQARTISAYGAERGVAIVPEIDTPGHMAAAFALLEAQHGTKWVDRIRSGENELDTSAPESLALAKKLYAEVQRTFPSSRTVHIGGDEWGDDVTAAQRVTWMNAMAAALDDREVWAWNDGIDRVAVGRLDPRIHVTYWSFDGDTEDAAERRERRARRASAVDLQQAGIDQLNYNSYYLYEVPTDLDPADSDYTVADLRENWSLRAWDGDSGSLLAAPMSGAAVAIWGEDLEDPPSDALLRWSAPHVTAMIETAAS

SEQ ID NO: 34 - protein, 445 aa, Mature polypeptide from Curtobacterium luteum
DTAVSAVTVTKVTASTTGTAVRTTLKVENTAPVRKPASSVWLYLSAGTEKYTLGRVAVKALSAGSSTSVTAVRGTPSRAAAGKYWVLACAGAYSAKQCRTSTATVTTKPTKRARPETGVMLDVARAYYPVALIKRYIDLLADDGGRFLHLHLTDDQNVGIESTVLGQTPANADLDHGVYTSRVTHRPFLSAAQARTISEYGAERGVTIVPEIDTPGHMAAAFALLEAQHGTKWVDRIRSGENELDTSAPESLVLAKKLYAEVQRTFPSSRTVHIGGDEWGDDVTAAHRVAWMNEMAATLGNREVWAWNDGIDRVAVGRLDPRIHVTYWSFDGDTEDAAERRERRARRASAVDLQQAGIDQLNYNSYYLYEVPTDLDPADSDYTVADLRENWSLRAWDGDSGSLLAAPMSGAAVAIWGEDLEDPPSDALLRWSAPHVTAMIETAAS

SEQ ID NO: 35 - protein, 458 aa, mature polypeptide from Curtobacterium oceanosedimentum
IGGSAGTADASGAPRLVVTKVTASSTTTSTRTTVRTTLTVKNTSVARKPAADAWLSLTAGSKRYTLGHVSVQSLAAGASATIHATHTAPPRAPAGKYAVLACTGAFSLSKCGTSATTVTTARATRARPDTGVMLDVARAYYPVALIEQYIALLADHGGRFLHLHLTDDQNVGIESEVLGQTLANADLRDGVYTSRITGRPFLSAAQAREISRYAAQRGIAIIPEIDTPGHMAAAFALLEAGHGKQWVDRIRSGESELDTSAPGSSALAARLLQEVTRTFPSSRTVHIGGDEWGDDVTADERVQWLNTMAAAVGNRAVWAWNDGIDRAAIGRLDPRIHVTYWSFDGDTEDATERRERRERRAGANDLYAAGIDLLNYNSYYLYEVPTDLDAADSEYTVADLRENWSLRTWDGDSGARLAGPTSGAAVAIWGEDLEAPPSDALLRWSAPHVLAMIETAGS

SEQ ID NO: 36 - protein, 450 aa, mature polypeptide from Curtobacterium leaf154
AGSTTSTVTVTQVTATTTASSTGTAVRTTLKIKNTAAVRKPASSAWLYLSAGTKKYTLGRVAVKALAAGSSTSVTAVRGTPSRATAGEYSVLACAGAYSAKQCRTSTATVTTKPTKRARPETGVMLDVARAYYPVALIKRYIDLLADDGGRFLHLHLTDDQNVGIESTVLGQTLANADLDEGVYTSRVTRRPFLSAAQARTISDYAARRGVAIVPEIDTPGHMTAAFDLLEAQHGTKWVDRIRSGENELDTSTPGSLALAKKLYAEVQRTFPASRTVHIGGDEWGDDVSAAERVAWMNAMAAALGNREVWAWNDGIDRVAVGRLDPRIHVTYWSFDGDTEDAAERRERRARRASAVDLQQAGIDMLNYNSYYLYEVPTDLDPADSEYTVADLRENWSLRTWDGDSGSLLAAPMSGAAVAIWGEDLEDPPSDALLRWSAPHVTAMIETAAS

SEQ ID NO: 37 - protein, 306 aa, GH20 catalytic domain from Curtobacterium flaccumfaciens
GVMLDVARAYYPVALIKRYIDLLADDGGRFLHLHLTDDQNVGIESTVLGQTPANADLDHGVYTSRVTHRPFLSAAQARTISAYGAERGVAIVPEIDTPGHMAAAFALLEAQHGTKWVDRIRSGENELDTSAPESLALAKKLYAEVQRTFPSSRTVHIGGDEWGDDVTAAQRVTWMNAMAAALDDREVWAWNDGIDRVAVGRLDPRIHVTYWSFDGDTEDAAERRERRARRASAVDLQQAGIDQLNYNSYYLYEVPTDLDPADSDYTVADLRENWSLRAWDGDSGSLLAAPMSGAAVAIWGEDLEDP

SEQ ID NO: 38 - protein, 306 aa, GH20 catatlytic domain from Curtobacterium luteum
GVMLDVARAYYPVALIKRYIDLLADDGGRFLHLHLTDDQNVGIESTVLGQTPANADLDHGVYTSRVTHRPFLSAAQARTISEYGAERGVTIVPEIDTPGHMAAAFALLEAQHGTKWVDRIRSGENELDTSAPESLVLAKKLYAEVQRTFPSSRTVHIGGDEWGDDVTAAHRVAWMNEMAATLGNREVWAWNDGIDRVAVGRLDPRIHVTYWSFDGDTEDAAERRERRARRASAVDLQQAGIDQLNYNSYYLYEVPTDLDPADSDYTVADLRENWSLRAWDGDSGSLLAAPMSGAAVAIWGEDLEDP

SEQ ID NO: 39 - protein, 304 aa, GH20 catatlytic domain from Curtobacterium oceanosedimentum
GVMLDVARAYYPVALIEQYIALLADHGGRFLHLHLTDDQNVGIESEVLGQTLANADLRDGVYTSRITGRPFLSAAQAREISRYAAQRGIAIIPEIDTPGHMAAAFALLEAGHGKQWVDRIRSGESELDTSAPGSSALAARLLQEVTRTFPSSRTVHIGGDEWGDDVTADERVQWLNTMAAAVGNRAVWAWNDGIDRAAIGRLDPRIHVTYWSFDGDTEDATERRERRERRAGANDLYAAGIDLLNYNSYYLYEVPTDLDAADSEYTVADLRENWSLRTWDGDSGARLAGPTSGAAVAIWGEDLE

SEQ ID NO: 40 - protein, 306 aa, GH20 catatlytic domain from Curtobacterium leaf154
GVMLDVARAYYPVALIKRYIDLLADDGGRFLHLHLTDDQNVGIESTVLGQTLANADLDEGVYTSRVTRRPFLSAAQARTISDYAARRGVAIVPEIDTPGHMTAAFDLLEAQHGTKWVDRIRSGENELDTSTPGSLALAKKLYAEVQRTFPASRTVHIGGDEWGDDVSAAERVAWMNAMAAALGNREVWAWNDGIDRVAVGRLDPRIHVTYWSFDGDTEDAAERRERRARRASAVDLQQAGIDMLNYNSYYLYEVPTDLDPADSEYTVADLRENWSLRTWDGDSGSLLAAPMSGAAVAIWGEDLEDP

SEQ ID NO: 41 - protein, 4 aa, Artificial
  Motif
  MISC_FEATURE (2)..(2): Xaa = Any natural amino acid
GXDE

SEQ ID NO: 42 - protein, 7 aa, Artificial
  Motif
ARAYYPV

SEQ ID NO: 43 - protein, 7 aa, Artificial
  Motif
AWNDGID

SEQ ID NO: 44 - protein, 7 aa, Artificial
  Motif
DDQNVGI

SEQ ID NO: 45 - protein, 5 aa, Artificial
  Motif
DPRIH

SEQ ID NO: 46 - protein, 7 aa, Artificial
  Motif
  MISC_FEATURE (1)..(1): Xaa = (Glu) E or (Gln) Q
  MISC_FEATURE (2)..(2): Xaa = (Asn) N or (Arg) R or (Ser) S or His (H) or Ala (A)
  MISC_FEATURE (3)..(3): Xaa = (Tyr) Y or (Val) V or (Phe) F or (leu) L
  MISC_FEATURE (4)..(4): Xaa = (Ala) A or (Gly) G or (Ser) S or (Thr) T or (Cys) C
  MISC_FEATURE (5)..(5): Xaa = (Ile) I or (Val) V or (Leu) L or (Phe) F
  MISC_FEATURE (6)..(6): Xaa = (Glu) E or (Ala) A or (Gln) Q or (Tyr) Y or (Asn) N
  MISC_FEATURE (7)..(7): Xaa = (Ser) S or (Asn) N
XXXXXXX